European Patent Application EP 4 600 270 A1, published August 13, 2025. Title: Anti-CD7 single domain antibody, a pharmaceutical composition and a kit for use in the diagnosis and/or therapy of cancer. Applicant: ImnoTech GmbH. Application EP. The sequence listing filed with the application follows.

SEQUENCE LISTING (25 sequences)

SEQ ID NO: 1 - protein, 240 aa, Homo sapiens
MAGPPRLLLLPLLLALARGLPGALAAQEVQQSPHCTTVPVGASVNITCSTSGGLRGIYLRQLGPQPQDIIYYEDGVVPTTDRRFRGRIDFSGSQDNLTITMHRLQLSDTGTYTCQAITEVNVYGSGTLVLVTEEQSQGWHRCSDAPPRASALPAPPTGSALPDPQTASALPDPPAASALPAALAVISFLLGLGLGVACVLARTQIKKLCSWRDKNSAACVVYEDMSHSRCNTLSSPNQYQ

SEQ ID NO: 2 - protein, 124 aa, Lama glama
QVQLQESGGGLVQAGGSLRLSCAASGRTFSDYLMGWFRQTPGKEREFVAAIYWNAGSTYYADSVKGRFTISRDNTKNTMYLQMNSLKPEDTAVYYCAAGQRGLAYARTYDYDYWGQGTQVTVSS

SEQ ID NO: 3 - protein, 117 aa, Lama glama
QVQLQESGGGLVQAGGSLRLSCAASGLTVSMYGMGWFRQAPGKEREFVADISRGGGSTSYTDSVKGRFTISRDNAKNTLYLQMNSLKPEDTAVYSCAARKYAHYEYWGQGTQVTVSS

SEQ ID NO: 4 - protein, 117 aa, Lama glama
QVQLQESGGGLVQAGDSLRLSCAASGLTVSSYGMGWFRQAPGKEREFVVDISRGGGSTSYADSVKGRFTIARDNAKNTLYLQMNSLKPEDTAVYSCAARKYAHYEYWGQGTQVTVSS

SEQ ID NO: 5 - protein, 117 aa, Lama glama
QVQLQESGGGLVQAGDSLRLSCAASGLTVSSYGMGWFRQAPGKEREFVADISRGGGSTSYADSVKGRFTISRDNAKNTLYLQMNSLKPEDTAVYSCAARKYAHYEYWGXGTQVTVSS

SEQ ID NO: 6 - protein, 124 aa, Lama glama
QVQLQESGGGLVQAGGSLRLSCAASGRTWSSYLMGWFRQTPGKEREFVAAIYWNAGSTYYSDSVKGRFTISRDNTKNTAYLQMNSLKPEDTAVYYCAAGQRGFAYARTYDYDYWGQGTQVTVSS

SEQ ID NO: 7 - protein, 117 aa, Lama glama
QVQLQESGGGLVQAGDSLRLSCAASGLTVSMYGMGWFRQAPGKEREFVADISRGGGSTSYTDSVKGRFTISRDNAKNTLYLQMNSLKPEDTAVYSCAARKYAHYEYRGQGTQVTVSS

SEQ ID NO: 8 - protein, 117 aa, Lama glama
QVQLQESGGGLVQTGDSLRLSCAASGLTVSSYGMGWFRQAPGKEREFVADISRGGGSTLYADSVKGRFTISRDNLKNTLYLQMNSLKPEDTAVYSCAARKYAEWNYWGQGTQVTVSS

SEQ ID NO: 9 - protein, 117 aa, Lama glama
QVQLQESGGGLVQAGDSLRLSCAASGLTVSSYGMGWFRQAPGKEREFVADISRGGGSTLYADSVKGRFTISRDNGKNTLYLQINSLKPEDTAVYSCAARKYAEWDYWGQGTQVTVSS

SEQ ID NO: 10 - protein, 124 aa, Lama glama
QVQLQESGGGLVQAGASLRLSCSASGRTFSDYLMGWFRQTPGKEREFVAAIYWNAGSTYYADSVKGRFTISRDNTKNTAYLQMNSLKPEDTAVYYCAAGQRGLAYARTYDYDYWGQGTQVTVSS

SEQ ID NO: 11 - protein, 124 aa, Lama glama
QVQLQESGGGLVQPGGSLRLSCAASGRTFSDYLMGWFRXTPGKEREFVAAIYWNAGSTYYADSVKGRFTISRDNTKNTVYLQMNSLKPEDTAVYYCAAGQRGLAYARTYDYDYWGQGTQVTVSS

SEQ ID NO: 12 - protein, 117 aa, Lama glama
QVQLQESGGGLVQAGDSLRLSCAASGLTVSSYGMGWFRQAPGKEREFVADISRGGGSTLYADSVKGRFTISRDNAKNTLYLQINSLKPEDTAVYSCAARKYAEWDYWGQGTQVTVSS

SEQ ID NO: 13 - protein, 115 aa, Lama glama
QVQLQESGGGLVQSGGSLRLSCAASRRIFEINVMGWYRQAPEKQRELVGTITSFGGTNYADSVKGRFTISADYAKNTMYLQMNSLNPEDTAVYYCNAHYFSNDYWGQGTQVTVSS

SEQ ID NO: 14 - protein, 8 aa, Lama glama
GRTFSDYL

SEQ ID NO: 15 - protein, 8 aa, Lama glama
GLTVSMYG

SEQ ID NO: 16 - protein, 8 aa, Lama glama
GLTVSSYG

SEQ ID NO: 17 - protein, 8 aa, Lama glama
RRIFEINV

SEQ ID NO: 18 - protein, 8 aa, Lama glama
IYWNAGST

SEQ ID NO: 19 - protein, 8 aa, Lama glama
ISRGGGST

SEQ ID NO: 20 - protein, 7 aa, Lama glama
ITSFGGT

SEQ ID NO: 21 - protein, 17 aa, Lama glama
AAGQRGLAYARTYDYDY

SEQ ID NO: 22 - protein, 10 aa, Lama glama
AARKYAHYEY

SEQ ID NO: 23 - protein, 10 aa, Lama glama
AARKYAEWNY

SEQ ID NO: 24 - protein, 10 aa, Lama glama
AARKYAEWDY

SEQ ID NO: 25 - protein, 9 aa, Lama glama
NAHYFSNDY